European Patent Application EP 4 036 241 A9, published March 22, 2023. Title: CNS DELIVERY OF MRNA AND USES THEREOF. Applicant: SHIRE HUMAN GENETIC THERAPIES, INC. The sequence listing filed with the application follows.

SEQUENCE LISTING (15 sequences)

SEQ ID NO: 1 - RNA, 1511 nt, Homo sapiens
ggggacccgcggguuugcuauggcgaugagcagcggcggcagugguggcggcgucccggagcaggaggauuccgugcuguuccggcgcggcacaggccagagcgaugauucugacauuugggaugauacagcacugauaaaagcauaugauaaagcuguggcuucauuuaagcaugcucuaaagaauggugacauuugugaaacuucggguaaaccaaaaaccacaccuaaaagaaaaccugcuaagaagaauaaaagccaaaagaagaauacugcagcuuccuuacaacaguggaaaguuggggacaaauguucugccauuuggucagaagacgguugcauuuacccagcuaccauugcuucaauugauuuuaagagagaaaccuguguugugguuuacacuggauauggaaauagagaggagcaaaaucuguccgaucuacuuuccccaaucugugaaguagcuaauaauauagaacaaaaugcucaagagaaugaaaaugaaagccaaguuucaacagaugaaagugagaacuccaggucuccuggaaauaaaucagauaacaucaagcccaaaucugcuccauggaacucuuuucucccuccaccaccccccaugccagggccaagacugggaccaggaaagccaggucuaaaauucaauggcccaccaccgccaccgccaccaccaccaccccacuuacuaucaugcuggcugccuccauuuccuucuggaccaccaauaauucccccaccaccucccauauguccagauucucuugaugaugcugaugcuuugggaaguauguuaauuucaugguacaugaguggcuaucauacuggcuauuauauggguuucagacaaaaucaaaaagaaggaaggugcucacauuccuuaaauuaaggagaaaugcuggcauagagcagcacuaaaugacaccacuaaagaaacgaucagacagaucuggaaugugaagcguuauagaagauaacuggccucauuucuucaaaauaucaaguguugggaaagaaaaaaggaaguggaauggguaacucuucuugauuaaaaguuauguaauaaccaaaugcaaugugaaauauuuuacuggacucuauuuugaaaaaccaucuguaaaagacuggggugggggugggaggccagcacgguggugaggcaguugagaaaauuugaauguggauuagauuuugaaugauauuggauaauuauugguaauuuuuaugagcugugagaaggguguuguaguuuauaaaagacugucuuaauuugcauacuuaagcauuuaggaaugaaguguuagagugucuuaaaauguuucaaaugguuuaacaaaauguaugugaggcguauguggcaaaauguuacagaaucuaacugguggacauggcuguucauuguacuguuuuuuucuaucuucuauauguuuaaaaguauauaauaaaaauauuuaauuuuuuuuuaaaaaaaaaaaaaaaaaaacaaaaaaaaaaaa

SEQ ID NO: 2 - protein, 294 aa, Homo sapiens
MAMSSGGSGGGVPEQEDSVLFRRGTGQSDDSDIWDDTALIKAYDKAVASFKHALKNGDICETSGKPKTTPKRKPAKKNKSQKKNTAASLQQWKVGDKCSAIWSEDGCIYPATIASIDFKRETCVVVYTGYGNREEQNLSDLLSPICEVANNIEQNAQENENESQVSTDESENSRSPGNKSDNIKPKSAPWNSFLPPPPPMPGPRLGPGKPGLKFNGPPPPPPPPPPHLLSCWLPPFPSGPPIIPPPPPICPDSLDDADALGSMLISWYMSGYHTGYYMGFRQNQKEGRCSHSLN

SEQ ID NO: 3 - RNA, 885 nt, Artificial Sequence
  Description of Artificial Sequence: Synthetic polynucleotide
auggccaugagcagcggaggcagcggcggaggagugcccgagcaggaggacagcgugcuguucaggagaggcaccggccagagcgaugacagcgauaucugggacgauaccgcucugaucaaggccuacgacaaggccguggccagcuucaagcacgcccugaaaaacggcgacaucugcgagaccagcggcaagcccaagacaacccccaagagaaagcccgccaagaagaauaagagccagaaaaagaacaccgccgccagccugcagcaguggaaggugggcgacaagugcagcgccaucuggagcgaggacggcugcaucuaccccgccaccaucgccagcaucgacuucaagagagagaccugcguggucguguacaccggcuacggcaacagagaggagcagaaccugagcgaccugcugagccccauuugugagguggccaauaacaucgaacagaacgcccaggagaacgagaaugaaagccaggugagcaccgacgagagcgagaacagcagaucuccuggcaacaagagcgacaacaucaagccuaagucugccccuuggaacagcuuccugcccccuccuccacccaugcccggacccagacugggacccggaaaaccuggccugaaguucaacggaccaccucccccuccaccuccucccccaccucaucuccugagcugcuggcugccacccuuccccagcggacccccuaucaucccaccacccccucccaucugccccgacagccuggacgacgccgaugcccugggcagcaugcugaucagcugguacaugagcggcuaccacacaggauacuacaugggcuucagacagaaccagaaggagggcagaugcucccacucccugaacuga

SEQ ID NO: 4 - RNA, 885 nt, Artificial Sequence
  Description of Artificial Sequence: Synthetic polynucleotide
auggccaugagcagcggaggaagcggaggaggagugccagaacaggaagauagcgugcuguuucgccggggcaccggacaaucggacgacagcgauauuugggacgacacugcgcucaucaaggccuacgacaaggcgguggcuucguucaagcacgcucugaagaacggggauaucugugaaaccagcgguaaaccaaaaacuacgccgaaaaggaaacccgccaaaaagaacaagucacagaagaagaauaccgcugcgagcuugcagcaguggaaggugggcgacaagugcuccgcgauuuggucggaagaugguugcaucuacccggcaaccaucgccuccaucgacuuuaagcgggagacuugcgucguggucuacaccggauacggcaauagagaggaacagaaucugucagaccuucugucgccaaucugcgaggucgccaacaauaucgaacaaaacgcccaagagaacgagaaugagucccaaguguccacggacgaaucggaaaacucacgguccccugggaacaagucagauaacaucaagccuaaaucggcaccauggaacuccuuccugccgccuccgccuccgaugccgggcccgcgccugggaccggguaaacccgggcucaaguucaauggaccgccacccccacccccgccaccgccgccccaccuccucucgugcuggcugccgccguucccuuccggaccgccuaucauuccgccaccuccaccuaucugcccagacagccuggaugaugccgacgcauugggcuccaugcucaucucaugguacaugucgggauaccauacuggguauuacaugggcuucagacagaaccagaaggaaggacgcuguucccauagccugaacuag

SEQ ID NO: 5 - RNA, 1442 nt, Homo sapiens
ggggccccacgcugcgcacccgcggguuugcuauggcgaugagcagcggcggcagugguggcggcgucccggagcaggaggauuccgugcuguuccggcgcggcacaggccagagcgaugauucugacauuugggaugauacagcacugauaaaagcauaugauaaagcuguggcuucauuuaagcaugcucuaaagaauggugacauuugugaaacuucggguaaaccaaaaaccacaccuaaaagaaaaccugcuaagaagaauaaaagccaaaagaagaauacugcagcuuccuuacaacaguggaaaguuggggacaaauguucugccauuuggucagaagacgguugcauuuacccagcuaccauugcuucaauugauuuuaagagagaaaccuguguugugguuuacacuggauauggaaauagagaggagcaaaaucuguccgaucuacuuuccccaaucugugaaguagcuaauaauauagaacagaaugcucaagagaaugaaaaugaaagccaaguuucaacagaugaaagugagaacuccaggucuccuggaaauaaaucagauaacaucaagcccaaaucugcuccauggaacucuuuucucccuccaccaccccccaugccagggccaagacugggaccaggaaagccaggucuaaaauucaauggcccaccaccgccaccgccaccaccaccaccccacuuacuaucaugcuggcugccuccauuuccuucuggaccaccaauaauucccccaccaccucccauauguccagauucucuugaugaugcugaugcuuugggaaguauguuaauuucaugguacaugaguggcuaucauacuggcuauuauauggaaaugcuggcauagagcagcacuaaaugacaccacuaaagaaacgaucagacagaucuggaaugugaagcguuauagaagauaacuggccucauuucuucaaaauaucaaguguugggaaagaaaaaaggaaguggaauggguaacucuucuugauuaaaaguuauguaauaaccaaaugcaaugugaaauauuuuacuggacucuauuuugaaaaaccaucuguaaaagacugaggugggggugggaggccagcacgguggugaggcaguugagaaaauuugaauguggauuagauuuugaaugauauuggauaauuauugguaauuuuaugagcugugagaaggguguuguaguuuauaaaagacugucuuaauuugcauacuuaagcauuuaggaaugaaguguuagagugucuuaaaauguuucaaaugguuuaacaaaauguaugugaggcguauguggcaaaauguuacagaaucuaacugguggacauggcuguucauuguacuguuuuuuucuaucuucuauauguuuaaaaguauauaauaaaaauauuuaauuuuuuuuuaaaaa

SEQ ID NO: 6 - protein, 282 aa, Homo sapiens
MAMSSGGSGGGVPEQEDSVLFRRGTGQSDDSDIWDDTALIKAYDKAVASFKHALKNGDICETSGKPKTTPKRKPAKKNKSQKKNTAASLQQWKVGDKCSAIWSEDGCIYPATIASIDFKRETCVVVYTGYGNREEQNLSDLLSPICEVANNIEQNAQENENESQVSTDESENSRSPGNKSDNIKPKSAPWNSFLPPPPPMPGPRLGPGKPGLKFNGPPPPPPPPPPHLLSCWLPPFPSGPPIIPPPPPICPDSLDDADALGSMLISWYMSGYHTGYYMEMLA

SEQ ID NO: 7 - RNA, 140 nt, Artificial Sequence
  Description of Artificial Sequence: Synthetic polynucleotide
ggacagaucgccuggagacgccauccacgcuguuuugaccuccauagaagacaccgggaccgauccagccuccgcggccgggaacggugcauuggaacgcggauuccccgugccaagagugacucaccguccuugacacg

SEQ ID NO: 8 - RNA, 105 nt, Artificial Sequence
  Description of Artificial Sequence: Synthetic polynucleotide
cggguggcaucccugugaccccuccccagugccucuccuggcccuggaaguugccacuccagugcccaccagccuuguccuaauaaaauuaaguugcaucaagcu

SEQ ID NO: 9 - RNA, 105 nt, Artificial Sequence
  Description of Artificial Sequence: Synthetic polynucleotide
ggguggcaucccugugaccccuccccagugccucuccuggcccuggaaguugccacuccagugcccaccagccuuguccuaauaaaauuaaguugcaucaaagcu

SEQ ID NO: 10 - RNA, 1130 nt, Artificial Sequence
  Description of Artificial Sequence: Synthetic polynucleotide
ggacagaucgccuggagacgccauccacgcuguuuugaccuccauagaagacaccgggaccgauccagccuccgcggccgggaacggugcauuggaacgcggauuccccgugccaagagugacucaccguccuugacacgauggccaugagcagcggaggcagcggcggaggagugcccgagcaggaggacagcgugcuguucaggagaggcaccggccagagcgaugacagcgauaucugggacgauaccgcucugaucaaggccuacgacaaggccguggccagcuucaagcacgcccugaaaaacggcgacaucugcgagaccagcggcaagcccaagacaacccccaagagaaagcccgccaagaagaauaagagccagaaaaagaacaccgccgccagccugcagcaguggaaggugggcgacaagugcagcgccaucuggagcgaggacggcugcaucuaccccgccaccaucgccagcaucgacuucaagagagagaccugcguggucguguacaccggcuacggcaacagagaggagcagaaccugagcgaccugcugagccccauuugugagguggccaauaacaucgaacagaacgcccaggagaacgagaaugaaagccaggugagcaccgacgagagcgagaacagcagaucuccuggcaacaagagcgacaacaucaagccuaagucugccccuuggaacagcuuccugcccccuccuccacccaugcccggacccagacugggacccggaaaaccuggccugaaguucaacggaccaccucccccuccaccuccucccccaccucaucuccugagcugcuggcugccacccuuccccagcggacccccuaucaucccaccacccccucccaucugccccgacagccuggacgacgccgaugcccugggcagcaugcugaucagcugguacaugagcggcuaccacacaggauacuacaugggcuucagacagaaccagaaggagggcagaugcucccacucccugaacugacggguggcaucccugugaccccuccccagugccucuccuggcccuggaaguugccacuccagugcccaccagccuuguccuaauaaaauuaaguugcaucaagcu

SEQ ID NO: 11 - RNA, 1130 nt, Artificial Sequence
  Description of Artificial Sequence: Synthetic polynucleotide
ggacagaucgccuggagacgccauccacgcuguuuugaccuccauagaagacaccgggaccgauccagccuccgcggccgggaacggugcauuggaacgcggauuccccgugccaagagugacucaccguccuugacacgauggccaugagcagcggaggcagcggcggaggagugcccgagcaggaggacagcgugcuguucaggagaggcaccggccagagcgaugacagcgauaucugggacgauaccgcucugaucaaggccuacgacaaggccguggccagcuucaagcacgcccugaaaaacggcgacaucugcgagaccagcggcaagcccaagacaacccccaagagaaagcccgccaagaagaauaagagccagaaaaagaacaccgccgccagccugcagcaguggaaggugggcgacaagugcagcgccaucuggagcgaggacggcugcaucuaccccgccaccaucgccagcaucgacuucaagagagagaccugcguggucguguacaccggcuacggcaacagagaggagcagaaccugagcgaccugcugagccccauuugugagguggccaauaacaucgaacagaacgcccaggagaacgagaaugaaagccaggugagcaccgacgagagcgagaacagcagaucuccuggcaacaagagcgacaacaucaagccuaagucugccccuuggaacagcuuccugcccccuccuccacccaugcccggacccagacugggacccggaaaaccuggccugaaguucaacggaccaccucccccuccaccuccucccccaccucaucuccugagcugcuggcugccacccuuccccagcggacccccuaucaucccaccacccccucccaucugccccgacagccuggacgacgccgaugcccugggcagcaugcugaucagcugguacaugagcggcuaccacacaggauacuacaugggcuucagacagaaccagaaggagggcagaugcucccacucccugaacugaggguggcaucccugugaccccuccccagugccucuccuggcccuggaaguugccacuccagugcccaccagccuuguccuaauaaaauuaaguugcaucaaagcu

SEQ ID NO: 12 - DNA, 500 bp, Artificial Sequence
  Description of Artificial Sequence: Synthetic polynucleotide
  misc_feature (1)..(500): This sequence may encompass 10-500 nucleotides
  See specification as filed for detailed description of substitutions and preferred embodiments
aaaaaaaaaaaaaaaaaaaaaaaaaaaaaaaaaaaaaaaaaaaaaaaaaaaaaaaaaaaaaaaaaaaaaaaaaaaaaaaaaaaaaaaaaaaaaaaaaaaaaaaaaaaaaaaaaaaaaaaaaaaaaaaaaaaaaaaaaaaaaaaaaaaaaaaaaaaaaaaaaaaaaaaaaaaaaaaaaaaaaaaaaaaaaaaaaaaaaaaaaaaaaaaaaaaaaaaaaaaaaaaaaaaaaaaaaaaaaaaaaaaaaaaaaaaaaaaaaaaaaaaaaaaaaaaaaaaaaaaaaaaaaaaaaaaaaaaaaaaaaaaaaaaaaaaaaaaaaaaaaaaaaaaaaaaaaaaaaaaaaaaaaaaaaaaaaaaaaaaaaaaaaaaaaaaaaaaaaaaaaaaaaaaaaaaaaaaaaaaaaaaaaaaaaaaaaaaaaaaaaaaaaaaaaaaaaaaaaaaaaaaaaaaaaaaaaaaaaaaaaaaaaaaaaaaaaaaaaaaaaaaaaaaaaaaaaaaaaaaa

SEQ ID NO: 13 - DNA, 300 bp, Artificial Sequence
  Description of Artificial Sequence: Synthetic polynucleotide
  misc_feature (1)..(300): This sequence may encompass 10-300 nucleotides
  See specification as filed for detailed description of substitutions and preferred embodiments
aaaaaaaaaaaaaaaaaaaaaaaaaaaaaaaaaaaaaaaaaaaaaaaaaaaaaaaaaaaaaaaaaaaaaaaaaaaaaaaaaaaaaaaaaaaaaaaaaaaaaaaaaaaaaaaaaaaaaaaaaaaaaaaaaaaaaaaaaaaaaaaaaaaaaaaaaaaaaaaaaaaaaaaaaaaaaaaaaaaaaaaaaaaaaaaaaaaaaaaaaaaaaaaaaaaaaaaaaaaaaaaaaaaaaaaaaaaaaaaaaaaaaaaaaaaaaaaaaaaaaaaaaaaaaaaaaaaaaaaaaaaaaaaaaaaaaaaaaaaa

SEQ ID NO: 14 - DNA, 200 bp, Artificial Sequence
  Description of Artificial Sequence: Synthetic polynucleotide
  misc_feature (1)..(200): This sequence may encompass 10-200 nucleotides
  See specification as filed for detailed description of substitutions and preferred embodiments
cccccccccccccccccccccccccccccccccccccccccccccccccccccccccccccccccccccccccccccccccccccccccccccccccccccccccccccccccccccccccccccccccccccccccccccccccccccccccccccccccccccccccccccccccccccccccccccccccccccccc

SEQ ID NO: 15 - DNA, 250 bp, Artificial Sequence
  Description of Artificial Sequence: Synthetic polynucleotide
  See specification as filed for detailed description of substitutions and preferred embodiments
aaaaaaaaaaaaaaaaaaaaaaaaaaaaaaaaaaaaaaaaaaaaaaaaaaaaaaaaaaaaaaaaaaaaaaaaaaaaaaaaaaaaaaaaaaaaaaaaaaaaaaaaaaaaaaaaaaaaaaaaaaaaaaaaaaaaaaaaaaaaaaaaaaaaaaaaaaaaaaaaaaaaaaaaaaaaaaaaaaaaaaaaaaaaaaaaaaaaaaaaaaaaaaaaaaaaaaaaaaaaaaaaaaaaaaaaaaaaaaaaaaaaaaaaaa